European Patent Specification EP 3 978 531 B1, published July 29, 2026. Title: ANTI-TIM-3 ANTIBODIES AND COMPOSITIONS. Applicant: SYMPHOGEN A/S. Application Not yet assigned. The sequence listing filed with the application follows.

SEQUENCE LISTING (240 sequences)

SEQ ID NO: 1 - DNA, 360 bp, Artificial Sequence
  source: /note="Description of Artificial Sequence: Synthetic polynucleotide"
caggtgcagctacagcagtcgggcccaggactggtgaagccttcacagaccctgtccctcacctgcactgtctctggtggctccatcagcagtggtggttactactggagttggacccgtcagcacccagggatgggcctggagtggattggatacatctcttacagtgggagtatctattacactccgtccctcaagagtcgacttaccatatcagtggacacgtctaagaaccagttctccctgaagctgagctctgtgactgccgcggacacggccgtatattactgtgcgagtttggattcctggggatctaaccgtgactactggggccagggaaccctggtcaccgtctcgagt

SEQ ID NO: 2 - DNA, 321 bp, Artificial Sequence
  source: /note="Description of Artificial Sequence: Synthetic polynucleotide"
gaaattgtgttgacgcagtctccagccaccctgtctttgtctccaggggaaagagccaccctctcctgcagggccagtcagagtgttagcagctacttagcctggtaccaacagaaacctggccaggctcccaggctcctcatctatgatgcatccaacagggccactggcatcccagccaggttcagtggcagtgggtctgggacagacttcactctcaccatcagcagcctagagcctgaagattttgcagtttattactgtcagcagcgtagcaactggccgctcactttcggcggagggaccaaggtggagattaag

SEQ ID NO: 3 - protein, 120 aa, Artificial Sequence
  source: /note="Description of Artificial Sequence: Synthetic polypeptide"
QVQLQQSGPGLVKPSQTLSLTCTVSGGSISSGGYYWSWTRQHPGMGLEWIGYISYSGSIYYTPSLKSRLTISVDTSKNQFSLKLSSVTAADTAVYYCASLDSWGSNRDYWGQGTLVTVSS

SEQ ID NO: 4 - protein, 107 aa, Artificial Sequence
  source: /note="Description of Artificial Sequence: Synthetic polypeptide"
EIVLTQSPATLSLSPGERATLSCRASQSVSSYLAWYQQKPGQAPRLLIYDASNRATGIPARFSGSGSGTDFTLTISSLEPEDFAVYYCQQRSNWPLTFGGGTKVEIK

SEQ ID NO: 5 - protein, 330 aa, Artificial Sequence
  source: /note="Description of Artificial Sequence: Synthetic polypeptide"
ASTKGPSVFPLAPSSKSTSGGTAALGCLVKDYFPEPVTVSWNSGALTSGVHTFPAVLQSSGLYSLSSVVTVPSSSLGTQTYICNVNHKPSNTKVDKRVEPKSCDKTHTCPPCPAPELLGGPSVFLFPPKPKDTLMISRTPEVTCVVVDVSHEDPEVKFNWYVDGVEVHNAKTKPREEQYNSTYRVVSVLTVLHQDWLNGKEYKCKVSNKALPAPIEKTISKAKGQPREPQVYTLPPSREEMTKNQVSLTCLVKGFYPSDIAVEWESNGQPENNYKTTPPVLDSDGSFFLYSKLTVDKSRWQQGNVFSCSVMHEALHNHYTQKSLSLSPGK

SEQ ID NO: 6 - protein, 107 aa, Artificial Sequence [sequence omitted]

SEQ ID NO: 7 - protein, 10 aa, Artificial Sequence
  source: /note="Description of Artificial Sequence: Synthetic peptide"
GGSISSGGYY

SEQ ID NO: 8 - protein, 7 aa, Artificial Sequence
  source: /note="Description of Artificial Sequence: Synthetic peptide"
ISYSGSI

SEQ ID NO: 9 - protein, 14 aa, Artificial Sequence
  source: /note="Description of Artificial Sequence: Synthetic peptide"
CASLDSWGSNRDYW

SEQ ID NO: 10 - protein, 6 aa, Artificial Sequence
  source: /note="Description of Artificial Sequence: Synthetic peptide"
QSVSSY

SEQ ID NO: 11 - protein, 3 aa, Artificial Sequence
  source: /note="Description of Artificial Sequence: Synthetic peptide"
DAS

SEQ ID NO: 12 - protein, 11 aa, Artificial Sequence [sequence omitted]

SEQ ID NO: 13 - DNA, 360 bp, Artificial Sequence
  source: /note="Description of Artificial Sequence: Synthetic polynucleotide"
caggtgcagctgcaggagagtggccccggactggtcaagccttcacagactctgagcctgacctgcacagtgtctggcggaagtatcagctccgggggttactattggagctggacccgacagcacccaggaatgggtctggaatggatcgggtacatttcatatagcggctccatctactatacaccctcactgaaaagcaggctgaccatttccgtggacacatctaagaaccagttcagcctgaaactgtctagtgtgacagccgctgatactgcagtctactattgtgcctccctggactcttggggcagtaatagagattactggggccagggaactctggtcaccgtctcgagt

SEQ ID NO: 14 - DNA, 321 bp, Artificial Sequence
  source: /note="Description of Artificial Sequence: Synthetic polynucleotide"
gagatcgtgctgactcagtccccagccaccctgtcactgagcccaggagaacgagcaaccctgtcttgcagggcctcccagtctgtcagctcctacctggcttggtatcagcagaagcccgggcaggcacctcgactgctgatctacgacgccagtaacagagctaccggtattcccgcccgcttcagtggttcaggcagcggaacagactttaccctgacaatctctagtctggagcctgaagatttcgccgtgtactattgtcagcagaggtctaattggccactgacatttggcggagggactaaggtcgagatcaag

SEQ ID NO: 15 - protein, 120 aa, Artificial Sequence
  source: /note="Description of Artificial Sequence: Synthetic polypeptide"
QVQLQESGPGLVKPSQTLSLTCTVSGGSISSGGYYWSWTRQHPGMGLEWIGYISYSGSIYYTPSLKSRLTISVDTSKNQFSLKLSSVTAADTAVYYCASLDSWGSNRDYWGQGTLVTVSS

SEQ ID NO: 16 - DNA, 990 bp, Artificial Sequence
  source: /note="Description of Artificial Sequence: Synthetic polynucleotide"
gcctccaccaagggcccatcggtcttccccctggcaccctcctccaagagcacctctgggggcacagcggccctgggctgcctggtcaaggactacttccccgaaccggtgacggtgtcgtggaactcaggcgccctgaccagcggcgtgcacaccttcccggctgtcctacagtcctcaggactctactccctcagcagcgtggtgaccgtgccctccagcagcttgggcacccagacctacatctgcaacgtgaatcacaagcccagcaacaccaaggtggacaagagagttgagcccaaatcttgtgacaaaactcacacatgcccaccgtgcccagcacctgaagccgccgggggaccgtcagtcttcctcttccccccaaaacccaaggacaccctcatgatctcccggacccctgaggtcacatgcgtggtggtggacgtgagccacgaagaccctgaggtcaagttcaactggtacgtggacggcgtggaggtgcataatgccaagacaaagccgcgggaggagcagtacaacagcacgtaccgtgtggtcagcgtcctcaccgtcctgcaccaggactggctgaatggcaaggagtacaagtgcaaggtctccaacaaagccctcccagcccccatcgagaaaaccatctccaaagccaaagggcagccccgagaaccacaggtgtacaccctgcccccatcccgggaggagatgaccaagaaccaggtcagcctgacctgcctggtcaaaggcttctatcccagcgacatcgccgtggagtgggagagcaatgggcagccggagaacaactacaagaccacgcctcccgtgctggactccgacggctccttcttcctctatagcaagctcaccgtggacaagagcaggtggcagcaggggaacgtcttctcatgctccgtgatgcatgaggctctgcacaaccactacacgcagaagagcctctccctgtccccgggtaaa

SEQ ID NO: 17 - DNA, 1596 bp, Artificial Sequence
  source: /note="Description of Artificial Sequence: Synthetic polynucleotide"
gcctccaccaagggcccatcggtcttccccctggcaccctcctccaagagcacctctgggggcacagcggccctgggctgcctggtcaaggactacttccccgaaccggtgacggtgtcgtggaactcaggcgccctgaccagcggcgtgcacaccttcccggctgtcctacagtcctcaggactctactccctcagcagcgtggtgaccgtgccctccagcagcttgggcacccagacctacatctgcaacgtgaatcacaagcccagcaacaccaaggtggacaagagagttggtgagaggccagcacagggagggagggtgtctgctggaagccaggctcagcgctcctgcctggacgcatcccggctatgcagtcccagtccagggcagcaaggcaggccccgtctgcctcttcacccggaggcctctgcccgccccactcatgctcagggagagggtcttctggctttttccccaggctctgggcaggcacaggctaggtgcccctaacccaggccctgcacacaaaggggcaggtgctgggctcagacctgccaagagccatatccgggaggaccctgcccctgacctaagcccaccccaaaggccaaactctccactccctcagctcggacaccttctctcctcccagattccagtaactcccaatcttctctctgcagagcccaaatcttgtgacaaaactcacacatgcccaccgtgcccaggtaagccagcccaggcctcgccctccagctcaaggcgggacaggtgccctagagtagcctgcatccagggacaggccccagccgggtgctgacacgtccacctccatctcttcctcagcacctgaagccgccgggggaccgtcagtcttcctcttccccccaaaacccaaggacaccctcatgatctcccggacccctgaggtcacatgcgtggtggtggacgtgagccacgaagaccctgaggtcaagttcaactggtacgtggacggcgtggaggtgcataatgccaagacaaagccgcgggaggagcagtacaacagcacgtaccgtgtggtcagcgtcctcaccgtcctgcaccaggactggctgaatggcaaggagtacaagtgcaaggtctccaacaaagccctcccagcccccatcgagaaaaccatctccaaagccaaaggtgggacccgtggggtgcgagggccacatggacagaggccggctcggcccaccctctgccctgagagtgaccgctgtaccaacctctgtccctacagggcagccccgagaaccacaggtgtacaccctgcccccatcccgggaggagatgaccaagaaccaggtcagcctgacctgcctggtcaaaggcttctatcccagcgacatcgccgtggagtgggagagcaatgggcagccggagaacaactacaagaccacgcctcccgtgctggactccgacggctccttcttcctctatagcaagctcaccgtggacaagagcaggtggcagcaggggaacgtcttctcatgctccgtgatgcatgaggctctgcacaaccactacacgcagaagagcctctccctgtccccgggtaaa

SEQ ID NO: 18 - DNA, 981 bp, Artificial Sequence
  source: /note="Description of Artificial Sequence: Synthetic polynucleotide"
gcttccaccaagggcccatcggtcttccccctggcgccctgctccaggagcacctccgagagcacagccgccctgggctgcctggtcaaggactacttccccgaaccggtgacggtgtcgtggaactcaggcgccctgaccagcggcgtgcacaccttcccggctgtcctacagtcctcaggactctactccctcagcagcgtggtgaccgtgccctccagcagcttgggcacgaagacctacacctgcaacgtagatcacaagcccagcaacaccaaggtggacaagagagttgagtccaaatatggtcccccatgcccaccatgcccagcacctgagttcctggggggaccatcagtcttcctgttccccccaaaacccaaggacactctcatgatctcccggacccctgaggtcacgtgcgtggtggtggacgtgagccaggaagaccccgaggtccagttcaactggtacgtggatggcgtggaggtgcataatgccaagacaaagccgcgggaggagcagttcaacagcacgtaccgtgtggtcagcgtcctcaccgtcctgcaccaggactggctgaacggcaaggagtacaagtgcaaggtctccaacaaaggcctcccgtcctccatcgagaaaaccatctccaaagccaaagggcagccccgagagccacaggtgtacaccctgcccccatcccaggaggagatgaccaagaaccaggtcagcctgacctgcctggtcaaaggcttctaccccagcgacatcgccgtggagtgggagagcaatgggcagccggagaacaactacaagaccacgcctcccgtgctggactccgacggctccttcttcctctacagcaggctcaccgtggacaagagcaggtggcaggaggggaatgtcttctcatgctccgtgatgcatgaggctctgcacaaccactacacacagaagagcctctccctgtctctgggtaaa

SEQ ID NO: 19 - DNA, 1588 bp, Artificial Sequence
  source: /note="Description of Artificial Sequence: Synthetic polynucleotide"
gcttccaccaagggcccatcggtcttccccctggcgccctgctccaggagcacctccgagagcacagccgccctgggctgcctggtcaaggactacttccccgaaccggtgacggtgtcgtggaactcaggcgccctgaccagcggcgtgcacaccttcccggctgtcctacagtcctcaggactctactccctcagcagcgtggtgaccgtgccctccagcagcttgggcacgaagacctacacctgcaacgtagatcacaagcccagcaacaccaaggtggacaagagagttggtgagaggccagcacagggagggagggtgtctgctggaagccaggctcagccctcctgcctggacgcaccccggctgtgcagccccagcccagggcagcaaggcaggccccatctgtctcctcacccggaggcctctgaccaccccactcatgctcagggagagggtcttctggatttttccaccaggctccgggcagccacaggctggatgcccctaccccaggccctgagcatacaggggcaggtgctgcgctcagacctgccaagagccatatccgggaggaccctgcccctgacctaagcccaccccaaaggccaaactctccactccctcagctcagacaccttctctcctcccagatctgagtaactcccaatcttctctctgcagagtccaaatatggtcccccatgcccaccatgcccaggtaagccaacccaggcctcgccctccagctcaaggcgggacaggtgccctagagtagcctgcatccagggacaggccccagccgggtgctgacgcatccacctccatctcttcctcagcacctgagttcctggggggaccatcagtcttcctgttccccccaaaacccaaggacactctcatgatctcccggacccctgaggtcacgtgcgtggtggtggacgtgagccaggaagaccccgaggtccagttcaactggtacgtggatggcgtggaggtgcataatgccaagacaaagccgcgggaggagcagttcaacagcacgtaccgtgtggtcagcgtcctcaccgtcctgcaccaggactggctgaacggcaaggagtacaagtgcaaggtctccaacaaaggcctcccgtcctccatcgagaaaaccatctccaaagccaaaggtgggacccacggggtgcgagggccacatggacagaggtcagctcggcccaccctctgccctgggagtgaccgctgtgccaacctctgtccctacagggcagccccgagagccacaggtgtacaccctgcccccatcccaggaggagatgaccaagaaccaggtcagcctgacctgcctggtcaaaggcttctaccccagcgacatcgccgtggagtgggagagcaatgggcagccggagaacaactacaagaccacgcctcccgtgctggactccgacggctccttcttcctctacagcaggctcaccgtggacaagagcaggtggcaggaggggaatgtcttctcatgctccgtgatgcatgaggctctgcacaaccactacacacagaagagcctctccctgtctctgggtaaa

SEQ ID NO: 20 - DNA, 978 bp, Artificial Sequence
  source: /note="Description of Artificial Sequence: Synthetic polynucleotide"
gcctccaccaagggcccatcggtcttccccctggcgccctgctccaggagcacctccgagagcacagccgccctgggctgcctggtcaaggactacttccccgaaccggtgacggtgtcgtggaactcaggcgctctgaccagcggcgtgcacaccttcccagctgtcctacagtcctcaggactctactccctcagcagcgtggtgaccgtgccctccagcaacttcggcacccagacctacacctgcaacgtagatcacaagcccagcaacaccaaggtggacaagacagttgagcgcaaatgttgtgtcgagtgcccaccgtgcccagcaccacctgtggcaggaccgtcagtcttcctcttccccccaaaacccaaggacaccctcatgatctcccggacccctgaggtcacgtgcgtggtggtggacgtgagccacgaagaccccgaggtccagttcaactggtacgtggacggcgtggaggtgcataatgccaagacaaagccacgggaggagcagttcaacagcacgttccgtgtggtcagcgtcctcaccgttgtgcaccaggactggctgaacggcaaggagtacaagtgcaaggtctccaacaaaggcctcccagcccccatcgagaaaaccatctccaaaaccaaagggcagccccgagaaccacaggtgtacaccctgcccccatcccgggaggagatgaccaagaaccaggtcagcctgacctgcctggtcaaaggcttctaccccagcgacatcgccgtggagtgggagagcaatgggcagccggagaacaactacaagaccacacctcccatgctggactccgacggctccttcttcctctacagcaagctcaccgtggacaagagcaggtggcagcaggggaacgtcttctcatgctccgtgatgcatgaggctctgcacaaccactacacgcagaagagcctctccctgtctccgggtaaa

SEQ ID NO: 21 - DNA, 1585 bp, Artificial Sequence
  source: /note="Description of Artificial Sequence: Synthetic polynucleotide"
gcctccaccaagggcccatcggtcttccccctggcgccctgctccaggagcacctccgagagcacagccgccctgggctgcctggtcaaggactacttccccgaaccggtgacggtgtcgtggaactcaggcgctctgaccagcggcgtgcacaccttcccagctgtcctacagtcctcaggactctactccctcagcagcgtggtgaccgtgccctccagcaacttcggcacccagacctacacctgcaacgtagatcacaagcccagcaacaccaaggtggacaagacagttggtgagaggccagctcagggagggagggtgtctgctggaagccaggctcagccctcctgcctggacgcaccccggctgtgcagccccagcccagggcagcaaggcaggccccatctgtctcctcacccggaggcctctgcccgccccactcatgctcagggagagggtcttctggctttttccaccaggctccaggcaggcacaggctgggtgcccctaccccaggcccttcacacacaggggcaggtgcttggctcagacctgccaaaagccatatccgggaggaccctgcccctgacctaagccgaccccaaaggccaaactgtccactccctcagctcggacaccttctctcctcccagatccgagtaactcccaatcttctctctgcagagcgcaaatgttgtgtcgagtgcccaccgtgcccaggtaagccagcccaggcctcgccctccagctcaaggcgggacaggtgccctagagtagcctgcatccagggacaggccccagctgggtgctgacacgtccacctccatctcttcctcagcaccacctgtggcaggaccgtcagtcttcctcttccccccaaaacccaaggacaccctcatgatctcccggacccctgaggtcacgtgcgtggtggtggacgtgagccacgaagaccccgaggtccagttcaactggtacgtggacggcgtggaggtgcataatgccaagacaaagccacgggaggagcagttcaacagcacgttccgtgtggtcagcgtcctcaccgttgtgcaccaggactggctgaacggcaaggagtacaagtgcaaggtctccaacaaaggcctcccagcccccatcgagaaaaccatctccaaaaccaaaggtgggacccgcggggtatgagggccacatggacagaggccggctcggcccaccctctgccctgggagtgaccgctgtgccaacctctgtccctacagggcagccccgagaaccacaggtgtacaccctgcccccatcccgggaggagatgaccaagaaccaggtcagcctgacctgcctggtcaaaggcttctaccccagcgacatcgccgtggagtgggagagcaatgggcagccggagaacaactacaagaccacacctcccatgctggactccgacggctccttcttcctctacagcaagctcaccgtggacaagagcaggtggcagcaggggaacgtcttctcatgctccgtgatgcatgaggctctgcacaaccactacacgcagaagagcctctccctgtctccgggtaaa

SEQ ID NO: 22 - DNA, 321 bp, Artificial Sequence
  source: /note="Description of Artificial Sequence: Synthetic polynucleotide"
cgtacggtggctgcaccatctgtcttcatcttcccgccatctgatgagcagttgaaatctggaactgcctctgttgtgtgcctgctgaataacttctatcccagagaggccaaagtacagtggaaggtggataacgccctccaatcgggtaactcccaggagagtgtcacagagcaggacagcaaggacagcacctacagcctcagcagcaccctgacgctgagcaaagcagactacgagaaacacaaagtctacgcctgcgaagtcacccatcagggcctgagctcgcccgtcacaaagagcttcaacaggggagagtgt

SEQ ID NO: 23 - protein, 330 aa, Artificial Sequence
  source: /note="Description of Artificial Sequence: Synthetic polypeptide"
ASTKGPSVFPLAPSSKSTSGGTAALGCLVKDYFPEPVTVSWNSGALTSGVHTFPAVLQSSGLYSLSSVVTVPSSSLGTQTYICNVNHKPSNTKVDKRVEPKSCDKTHTCPPCPAPEAAGGPSVFLFPPKPKDTLMISRTPEVTCVVVDVSHEDPEVKFNWYVDGVEVHNAKTKPREEQYNSTYRVVSVLTVLHQDWLNGKEYKCKVSNKALPAPIEKTISKAKGQPREPQVYTLPPSREEMTKNQVSLTCLVKGFYPSDIAVEWESNGQPENNYKTTPPVLDSDGSFFLYSKLTVDKSRWQQGNVFSCSVMHEALHNHYTQKSLSLSPGK

SEQ ID NO: 24 - protein, 327 aa, Artificial Sequence
  source: /note="Description of Artificial Sequence: Synthetic polypeptide"
ASTKGPSVFPLAPCSRSTSESTAALGCLVKDYFPEPVTVSWNSGALTSGVHTFPAVLQSSGLYSLSSVVTVPSSSLGTKTYTCNVDHKPSNTKVDKRVESKYGPPCPPCPAPEFLGGPSVFLFPPKPKDTLMISRTPEVTCVVVDVSQEDPEVQFNWYVDGVEVHNAKTKPREEQFNSTYRVVSVLTVLHQDWLNGKEYKCKVSNKGLPSSIEKTISKAKGQPREPQVYTLPPSQEEMTKNQVSLTCLVKGFYPSDIAVEWESNGQPENNYKTTPPVLDSDGSFFLYSRLTVDKSRWQEGNVFSCSVMHEALHNHYTQKSLSLSLGK

SEQ ID NO: 25 - protein, 326 aa, Artificial Sequence
  source: /note="Description of Artificial Sequence: Synthetic polypeptide"
ASTKGPSVFPLAPCSRSTSESTAALGCLVKDYFPEPVTVSWNSGALTSGVHTFPAVLQSSGLYSLSSVVTVPSSNFGTQTYTCNVDHKPSNTKVDKTVERKCCVECPPCPAPPVAGPSVFLFPPKPKDTLMISRTPEVTCVVVDVSHEDPEVQFNWYVDGVEVHNAKTKPREEQFNSTFRVVSVLTVVHQDWLNGKEYKCKVSNKGLPAPIEKTISKTKGQPREPQVYTLPPSREEMTKNQVSLTCLVKGFYPSDIAVEWESNGQPENNYKTTPPMLDSDGSFFLYSKLTVDKSRWQQGNVFSCSVMHEALHNHYTQKSLSLSPGK

SEQ ID NO: 26 - DNA, 354 bp, Artificial Sequence
  source: /note="Description of Artificial Sequence: Synthetic polynucleotide"
caggtgcagctacagcagtctgggggaggcttggtacagcctggggggtccctgagactctcctgtgcagcctctggattcaccttaagcagctatgccatgagctgggtccgccaggctccagggaaggggctggagtgggtctcaggtattagtggtagtggtggtagcacatacaacgcagactccgtgaagggccggttcaccatctccagagacaattccaagaacacgctgtttctgcaaatgaacagcctgagagccgaggacacggccgtatattactgtgcgaaaatttttgggtcctactactttgactactggggccagggaaccctggtcacagtctcgagt

SEQ ID NO: 27 - DNA, 339 bp, Artificial Sequence
  source: /note="Description of Artificial Sequence: Synthetic polynucleotide"
gaaattgtgatgacacagtctccagactccctggctgtgtctctgggcgagagggccaccatcaactgcaagtccagccagagtgttttatacagctccaacaataagaactacttagcttggtaccagcagaaaccaggacagcctcctaagctgctcatttactggacatctacccgggaatccggggtccctaaccgattcagtggcagcgggtctgggacagatttcactctcaccatcagcagcctgcaggctgaagatgtggcagtttattactgtcagcaatattatagtggtcctccgacgttcggccaagggaccaaggtggaaatcaaa

SEQ ID NO: 28 - protein, 118 aa, Artificial Sequence
  source: /note="Description of Artificial Sequence: Synthetic polypeptide"
QVQLQQSGGGLVQPGGSLRLSCAASGFTLSSYAMSWVRQAPGKGLEWVSGISGSGGSTYNADSVKGRFTISRDNSKNTLFLQMNSLRAEDTAVYYCAKIFGSYYFDYWGQGTLVTVSS

SEQ ID NO: 29 - protein, 113 aa, Artificial Sequence
  source: /note="Description of Artificial Sequence: Synthetic polypeptide"
EIVMTQSPDSLAVSLGERATINCKSSQSVLYSSNNKNYLAWYQQKPGQPPKLLIYWTSTRESGVPNRFSGSGSGTDFTLTISSLQAEDVAVYYCQQYYSGPPTFGQGTKVEIK

SEQ ID NO: 30 - protein, 8 aa, Artificial Sequence
  source: /note="Description of Artificial Sequence: Synthetic peptide"
GFTLSSYA

SEQ ID NO: 31 - protein, 8 aa, Artificial Sequence
  source: /note="Description of Artificial Sequence: Synthetic peptide"
ISGSGGST

SEQ ID NO: 32 - protein, 13 aa, Artificial Sequence
  source: /note="Description of Artificial Sequence: Synthetic peptide"
CAKIFGSYYFDYW

SEQ ID NO: 33 - protein, 12 aa, Artificial Sequence
  source: /note="Description of Artificial Sequence: Synthetic peptide"
QSVLYSSNNKNY

SEQ ID NO: 34 - protein, 3 aa, Artificial Sequence
  source: /note="Description of Artificial Sequence: Synthetic peptide"
WTS

SEQ ID NO: 35 - protein, 11 aa, Artificial Sequence [sequence omitted]

SEQ ID NO: 36 - DNA, 377 bp, Artificial Sequence
  source: /note="Description of Artificial Sequence: Synthetic polynucleotide"
acgtgacagggcgcgcccaggtccagctgcaggagagcggtcccggactggtgaagccatcccagacactgagcctgacttgtactgtgagcggcggtagcatctccagcggcggctactattggtcctggatcaggcagcacccaggcaagggcctggagtggatcggctacatctactatagcggctctatctactataacccttccctgaagagccgggtgaccatctctgtggacacatccaagaatcagttctatctgaagctgtcttccgtgaccgccgctgatacagccgtgtactattgcgcctcactgatggtctggggggtcatgggcgattactgggggcagggcacactggtcacagtctcgagt

SEQ ID NO: 37 - DNA, 321 bp, Artificial Sequence
  source: /note="Description of Artificial Sequence: Synthetic polynucleotide"
gagattgtgctgacccagtctcccgccaccctgtctctgagtcctggcgagagagccaccctgagctgcagagcctctcagtccgtgtccagctatctggcctggtatcagcagaagcccggccaggctccccggctgctgatctacgatgcctccaatagagccaccggcatccctgccagattctccggctctggctctggcaccgactttaccctgaccatctccagcctggaacccgaggacttcgccgtgtactactgccagcagcggtccgactggcctcctacatttggccaaggcaccaaggtggaaatcaag

SEQ ID NO: 38 - protein, 120 aa, Artificial Sequence
  source: /note="Description of Artificial Sequence: Synthetic polypeptide"
QVQLQESGPGLVKPSQTLSLTCTVSGGSISSGGYYWSWIRQHPGKGLEWIGYIYYSGSIYYNPSLKSRVTISVDTSKNQFYLKLSSVTAADTAVYYCASLMVWGVMGDYWGQGTLVTVSS

SEQ ID NO: 39 - protein, 107 aa, Artificial Sequence
  source: /note="Description of Artificial Sequence: Synthetic polypeptide"
EIVLTQSPATLSLSPGERATLSCRASQSVSSYLAWYQQKPGQAPRLLIYDASNRATGIPARFSGSGSGTDFTLTISSLEPEDFAVYYCQQRSDWPPTFGQGTKVEIK

SEQ ID NO: 40 - protein, 10 aa, Artificial Sequence
  source: /note="Description of Artificial Sequence: Synthetic peptide"
GGSISSGGYY

SEQ ID NO: 41 - protein, 7 aa, Artificial Sequence
  source: /note="Description of Artificial Sequence: Synthetic peptide"
IYYSGSI

SEQ ID NO: 42 - protein, 14 aa, Artificial Sequence
  source: /note="Description of Artificial Sequence: Synthetic peptide"
CASLMVWGVMGDYW

SEQ ID NO: 43 - protein, 6 aa, Artificial Sequence
  source: /note="Description of Artificial Sequence: Synthetic peptide"
QSVSSY

SEQ ID NO: 44 - protein, 3 aa, Artificial Sequence
  source: /note="Description of Artificial Sequence: Synthetic peptide"
DAS

SEQ ID NO: 45 - protein, 11 aa, Artificial Sequence [sequence omitted]

SEQ ID NO: 46 - DNA, 345 bp, Artificial Sequence
  source: /note="Description of Artificial Sequence: Synthetic polynucleotide"
caggtcaccttgaaggagtggggcgcaggactgttgaggccctcggagaccctgtccctcacctgcgctgtctatggtgggtccttcagtggttactactggagctggatccgccagcccccagggaaggggctggagtggataggggaaatcaatcatagtggaagcaccaactacaacccgtccctcaagagtcgagtcaccatatcagtagacgcgaccaagaaacaattctccctgaagctgacctctgtgaccgccgcggacacggctgtgtattactgtgcgagatattgggagctccctgactactggggccagggcaccctggtcaccgtctcgagt

SEQ ID NO: 47 - DNA, 321 bp, Artificial Sequence
  source: /note="Description of Artificial Sequence: Synthetic polynucleotide"
gacatccagttgacccagtctccatcctccctgtctgcatctgtaggagacagagtcaccatcacttgccgggcaagtcagggcattagaaatgatttaggctggtatcagcagaaaccagggaaagcccctaagcgcctgatctatgctgcatccagtttgcaaagtggggtcccatcaaggttcagcggcagtggatctgggacagaattcactctcacaatcagcagcctgcagcctgaagattttgcaacttattactgtctacagcataatagttaccctccgacgttcggccaagggaccaaggtggaaatcaag

SEQ ID NO: 48 - protein, 115 aa, Artificial Sequence
  source: /note="Description of Artificial Sequence: Synthetic polypeptide"
QVTLKEWGAGLLRPSETLSLTCAVYGGSFSGYYWSWIRQPPGKGLEWIGEINHSGSTNYNPSLKSRVTISVDATKKQFSLKLTSVTAADTAVYYCARYWELPDYWGQGTLVTVSS

SEQ ID NO: 49 - protein, 107 aa, Artificial Sequence
  source: /note="Description of Artificial Sequence: Synthetic polypeptide"
DIQLTQSPSSLSASVGDRVTITCRASQGIRNDLGWYQQKPGKAPKRLIYAASSLQSGVPSRFSGSGSGTEFTLTISSLQPEDFATYYCLQHNSYPPTFGQGTKVEIK

SEQ ID NO: 50 - protein, 8 aa, Artificial Sequence
  source: /note="Description of Artificial Sequence: Synthetic peptide"
GGSFSGYY

SEQ ID NO: 51 - protein, 7 aa, Artificial Sequence
  source: /note="Description of Artificial Sequence: Synthetic peptide"
INHSGST

SEQ ID NO: 52 - protein, 11 aa, Artificial Sequence
  source: /note="Description of Artificial Sequence: Synthetic peptide"
CARYWELPDYW

SEQ ID NO: 53 - protein, 6 aa, Artificial Sequence
  source: /note="Description of Artificial Sequence: Synthetic peptide"
QGIRND

SEQ ID NO: 54 - protein, 3 aa, Artificial Sequence
  source: /note="Description of Artificial Sequence: Synthetic peptide"
AAS

SEQ ID NO: 55 - protein, 11 aa, Artificial Sequence [sequence omitted]

SEQ ID NO: 56 - DNA, 345 bp, Artificial Sequence
  source: /note="Description of Artificial Sequence: Synthetic polynucleotide"
cagatgcagctggtgcagtggggcgcaggactgttgaagccttcggagaccctgtccctcacctgcgctgtctatggtgggtccttcagtggttactactggagctggatccgccagcccccagggaaggggctggagtggattggggaaatcaatcatagtggaagcaccaactacaacccgtccctcaagagtcgagtcaccatgtcagttgacacgtccaagcaccagttctccctgaagctgagctctgtgaccgccgcggacacggctgtgtattactgtgcgagatggtgggagcttcctgactactggggccagggaaccctggtcaccgtctcgagt

SEQ ID NO: 57 - DNA, 321 bp, Artificial Sequence
  source: /note="Description of Artificial Sequence: Synthetic polynucleotide"
gaaattgtgttgacgcagtctccatcctccctgtctgcatctgtaggagacagagtcaccatcacttgccgggcaagtcagggcattagaaatgatttaggctggtatcagcagaaaccagggaaagcccctaagcgcctgatctatgctgcatccagtttgcaaagtggggtcccatcaaggttcagcggcagtggatctgggacagaattcactctcacaatcagcagcctgcagcctgaagattttgcaacttattactgtctacagcataatagttacccgtggacgttcggccaagggaccaaggtggaaatcaag

SEQ ID NO: 58 - protein, 115 aa, Artificial Sequence
  source: /note="Description of Artificial Sequence: Synthetic polypeptide"
QMQLVQWGAGLLKPSETLSLTCAVYGGSFSGYYWSWIRQPPGKGLEWIGEINHSGSTNYNPSLKSRVTMSVDTSKHQFSLKLSSVTAADTAVYYCARWWELPDYWGQGTLVTVSS

SEQ ID NO: 59 - protein, 107 aa, Artificial Sequence
  source: /note="Description of Artificial Sequence: Synthetic polypeptide"
EIVLTQSPSSLSASVGDRVTITCRASQGIRNDLGWYQQKPGKAPKRLIYAASSLQSGVPSRFSGSGSGTEFTLTISSLQPEDFATYYCLQHNSYPWTFGQGTKVEIK

SEQ ID NO: 60 - protein, 8 aa, Artificial Sequence
  source: /note="Description of Artificial Sequence: Synthetic peptide"
GGSFSGYY

SEQ ID NO: 61 - protein, 7 aa, Artificial Sequence
  source: /note="Description of Artificial Sequence: Synthetic peptide"
INHSGST

SEQ ID NO: 62 - protein, 11 aa, Artificial Sequence
  source: /note="Description of Artificial Sequence: Synthetic peptide"
CARWWELPDYW

SEQ ID NO: 63 - protein, 6 aa, Artificial Sequence
  source: /note="Description of Artificial Sequence: Synthetic peptide"
QGIRND

SEQ ID NO: 64 - protein, 3 aa, Artificial Sequence
  source: /note="Description of Artificial Sequence: Synthetic peptide"
AAS

SEQ ID NO: 65 - protein, 11 aa, Artificial Sequence [sequence omitted]

SEQ ID NO: 66 - DNA, 351 bp, Artificial Sequence
  source: /note="Description of Artificial Sequence: Synthetic polynucleotide"
cagatgcagctggtgcaatggggcgcaggactgttgaagccttcggagaccctgtccctcacctgcgctgtctatggtgggtccttcagtggttactactggagctggatccgccagcccccagggaaggggctggagtggattggggaaatcaatcatagtggaagcaccaactacaacccgtccctcaagagtcgagtcaccatatcagtagacacgtccaagaaccagttctccctgaagctgagctctgtgaccgccgcggacacggctgtgtattactgtgcgaggttttactatgctccgaactttgactactggggccagggcaccctggtcaccgtctcgagt

SEQ ID NO: 67 - DNA, 318 bp, Artificial Sequence
  source: /note="Description of Artificial Sequence: Synthetic polynucleotide"
gaaattgtgttgacgcagtctccttccaccctgtctgcatctgtaggagacagagtcaccatcacttgccgggccagtcagagtattagtagctggttggcctggtatcagcagaaaccagggacagcccctaagctcctgatctataaggcgtctagtttagaaagtggggtcccatcaaggttcagcggcagtggatctgggacagaattcactctcaccatcagcagcctgcagcctgatgattttgcaacttattactgccaacagtataatagttattccactttcggcggagggaccaaggtggagatcaaa

SEQ ID NO: 68 - protein, 117 aa, Artificial Sequence
  source: /note="Description of Artificial Sequence: Synthetic polypeptide"
QMQLVQWGAGLLKPSETLSLTCAVYGGSFSGYYWSWIRQPPGKGLEWIGEINHSGSTNYNPSLKSRVTISVDTSKNQFSLKLSSVTAADTAVYYCARFYYAPNFDYWGQGTLVTVSS

SEQ ID NO: 69 - protein, 106 aa, Artificial Sequence
  source: /note="Description of Artificial Sequence: Synthetic polypeptide"
EIVLTQSPSTLSASVGDRVTITCRASQSISSWLAWYQQKPGTAPKLLIYKASSLESGVPSRFSGSGSGTEFTLTISSLQPDDFATYYCQQYNSYSTFGGGTKVEIK

SEQ ID NO: 70 - protein, 8 aa, Artificial Sequence
  source: /note="Description of Artificial Sequence: Synthetic peptide"
GGSFSGYY

SEQ ID NO: 71 - protein, 7 aa, Artificial Sequence
  source: /note="Description of Artificial Sequence: Synthetic peptide"
INHSGST

SEQ ID NO: 72 - protein, 13 aa, Artificial Sequence
  source: /note="Description of Artificial Sequence: Synthetic peptide"
CARFYYAPNFDYW

SEQ ID NO: 73 - protein, 6 aa, Artificial Sequence
  source: /note="Description of Artificial Sequence: Synthetic peptide"
QSISSW

SEQ ID NO: 74 - protein, 3 aa, Artificial Sequence
  source: /note="Description of Artificial Sequence: Synthetic peptide"
KAS

SEQ ID NO: 75 - protein, 10 aa, Artificial Sequence [sequence omitted]

SEQ ID NO: 76 - DNA, 360 bp, Artificial Sequence
  source: /note="Description of Artificial Sequence: Synthetic polynucleotide"
caggtgcagctgcagcagtcgggcccaggactggtgaagccttcggagaccctgtccctcacctgcactgtctctggtggctccatcagcagtagtaattactactggggctggatccgccagcccccagggaaggggctggagtggattgggagtatctattatagtgggaacacctactacaacccgtccctcaagagtcgagtcaccatatccgtagacacgtccaagaaccagttctccctgaagctgagttctgtgaccgccgcagacacggctgtgtattactgtgcgagacagacagtggctggccccctctttgactactggggccagggaaccctggtcaccgtctcgagt

SEQ ID NO: 77 - DNA, 321 bp, Artificial Sequence
  source: /note="Description of Artificial Sequence: Synthetic polynucleotide"
gaaattgtgatgacgcagtctccttccaccctgtctgcatctgtaggagacagagtcaccatcacttgccgggccagtcagagtattagtagctggttggcctggtatcagcagaaaccagggaaagcccctaaggtcctgatctataaggcgtctagtttagaaagtggggtcccatcaaggttcagcggcagtggatctgggacagaactcactctcaccatcagcagcctgcagcctgatgattttgcaacttattactgccaacagtataatagttattcattcactttcggccctgggaccaaagtggatatcaag

SEQ ID NO: 78 - protein, 120 aa, Artificial Sequence
  source: /note="Description of Artificial Sequence: Synthetic polypeptide"
QVQLQQSGPGLVKPSETLSLTCTVSGGSISSSNYYWGWIRQPPGKGLEWIGSIYYSGNTYYNPSLKSRVTISVDTSKNQFSLKLSSVTAADTAVYYCARQTVAGPLFDYWGQGTLVTVSS

SEQ ID NO: 79 - protein, 107 aa, Artificial Sequence
  source: /note="Description of Artificial Sequence: Synthetic polypeptide"
EIVMTQSPSTLSASVGDRVTITCRASQSISSWLAWYQQKPGKAPKVLIYKASSLESGVPSRFSGSGSGTELTLTISSLQPDDFATYYCQQYNSYSFTFGPGTKVDIK

SEQ ID NO: 80 - protein, 10 aa, Artificial Sequence
  source: /note="Description of Artificial Sequence: Synthetic peptide"
GGSISSSNYY

SEQ ID NO: 81 - protein, 7 aa, Artificial Sequence
  source: /note="Description of Artificial Sequence: Synthetic peptide"
IYYSGNT

SEQ ID NO: 82 - protein, 14 aa, Artificial Sequence
  source: /note="Description of Artificial Sequence: Synthetic peptide"
CARQTVAGPLFDYW

SEQ ID NO: 83 - protein, 6 aa, Artificial Sequence
  source: /note="Description of Artificial Sequence: Synthetic peptide"
QSISSW

SEQ ID NO: 84 - protein, 3 aa, Artificial Sequence
  source: /note="Description of Artificial Sequence: Synthetic peptide"
KAS

SEQ ID NO: 85 - protein, 11 aa, Artificial Sequence [sequence omitted]

SEQ ID NO: 86 - DNA, 375 bp, Artificial Sequence
  source: /note="Description of Artificial Sequence: Synthetic polynucleotide"
caggtccagctggtgcaatctggggctgaggtgaagaagcctggggcctcagtgaaggtctcctgcaaggctgctggatacaccttaaccggctactatatgcactgggtgcgacaggcccctggacaaggccttgagtggatgggacggatcaaccctaacagtggtggctcaaacaatgcacagaagtttcagggcagggtcaccatgaccagggacacgtccatcagcacagcctacatggagctgagcaggctgagatctgacgacacggccgtgtattactgtgcgagagagggtcccctgtatagcagtggctggtacgagggtgcttttgatatctggggccaagggacaatggtcaccgtctcgagt

SEQ ID NO: 87 - DNA, 327 bp, Artificial Sequence
  source: /note="Description of Artificial Sequence: Synthetic polynucleotide"
gaaattgtgatgacgcagtctccttccaccctgtctgcatctgtaggagacagagtcaccatcacttgccgggccagtcagagtattagtagttggttggcctggtatcagcagaaaccagggaaagcccctaagctcctgatctataaggcgtctagtttagaaagtggggtcccatcaaggttcagcggcagtggatctgggacagaattcactctcaccatcagcagcctgcagcctgatgattttgcaacttattactgccaacagtataatagttattctccggggctcactttcggcggagggaccaaggtggagatcaag

SEQ ID NO: 88 - protein, 125 aa, Artificial Sequence
  source: /note="Description of Artificial Sequence: Synthetic polypeptide"
QVQLVQSGAEVKKPGASVKVSCKAAGYTLTGYYMHWVRQAPGQGLEWMGRINPNSGGSNNAQKFQGRVTMTRDTSISTAYMELSRLRSDDTAVYYCAREGPLYSSGWYEGAFDIWGQGTMVTVSS

SEQ ID NO: 89 - protein, 109 aa, Artificial Sequence
  source: /note="Description of Artificial Sequence: Synthetic polypeptide"
EIVMTQSPSTLSASVGDRVTITCRASQSISSWLAWYQQKPGKAPKLLIYKASSLESGVPSRFSGSGSGTEFTLTISSLQPDDFATYYCQQYNSYSPGLTFGGGTKVEIK

SEQ ID NO: 90 - protein, 8 aa, Artificial Sequence
  source: /note="Description of Artificial Sequence: Synthetic peptide"
GYTLTGYY

SEQ ID NO: 91 - protein, 8 aa, Artificial Sequence
  source: /note="Description of Artificial Sequence: Synthetic peptide"
INPNSGGS

SEQ ID NO: 92 - protein, 20 aa, Artificial Sequence
  source: /note="Description of Artificial Sequence: Synthetic peptide"
CAREGPLYSSGWYEGAFDIW

SEQ ID NO: 93 - protein, 6 aa, Artificial Sequence
  source: /note="Description of Artificial Sequence: Synthetic peptide"
QSISSW

SEQ ID NO: 94 - protein, 3 aa, Artificial Sequence
  source: /note="Description of Artificial Sequence: Synthetic peptide"
KAS

SEQ ID NO: 95 - protein, 13 aa, Artificial Sequence [sequence omitted]

SEQ ID NO: 96 - DNA, 372 bp, Artificial Sequence
  source: /note="Description of Artificial Sequence: Synthetic polynucleotide"
cagatgcagctacagcagtcaggtccaggactggtgaagccctcgcagaccctctcactcacctgtgccatctccggggacagtgtctctagcaacagtgctgcttggaactggatcaggcagtccccatcgagaggccttgagtggctgggaaggacatactacaggtccaagtggtattctgcttttgcagtatctgtgaaaagtcgaataaccatcaacccagacacatccaagaaccagttctccctgcagctgaactctgtgactcccgaggacacggctgtgtattactgtgcaagagagggtagcagtggctggtacggatacgtccaccactggggccagggcaccctggtcaccgtctcgagt

SEQ ID NO: 97 - DNA, 321 bp, Artificial Sequence
  source: /note="Description of Artificial Sequence: Synthetic polynucleotide"
gaaattgtgttgacgcagtctccagcttccctgtctgtatctctgggagaaactgtcaccatcgaatgtcgagcaagtgaggacatttacaatggtttagcatggtatcagcagaagccagggaaatctcctcagctcctgatctataatgcaaatagcttgcatactggggtcccatcacggttcagtggcagtggatctggtacacagtattctctcaagataaacagcctgcaatctgaagatgtcgcaagttatttctgtcaacagtattacgattatcctccgacgttcggccaagggaccaaggtggaaatcaaa

SEQ ID NO: 98 - protein, 124 aa, Artificial Sequence
  source: /note="Description of Artificial Sequence: Synthetic polypeptide"
QMQLQQSGPGLVKPSQTLSLTCAISGDSVSSNSAAWNWIRQSPSRGLEWLGRTYYRSKWYSAFAVSVKSRITINPDTSKNQFSLQLNSVTPEDTAVYYCAREGSSGWYGYVHHWGQGTLVTVSS

SEQ ID NO: 99 - protein, 107 aa, Artificial Sequence
  source: /note="Description of Artificial Sequence: Synthetic polypeptide"
EIVLTQSPASLSVSLGETVTIECRASEDIYNGLAWYQQKPGKSPQLLIYNANSLHTGVPSRFSGSGSGTQYSLKINSLQSEDVASYFCQQYYDYPPTFGQGTKVEIK

SEQ ID NO: 100 - protein, 10 aa, Artificial Sequence
  source: /note="Description of Artificial Sequence: Synthetic peptide"
GDSVSSNSAA

SEQ ID NO: 101 - protein, 9 aa, Artificial Sequence
  source: /note="Description of Artificial Sequence: Synthetic peptide"
TYYRSKWYS

SEQ ID NO: 102 - protein, 16 aa, Artificial Sequence
  source: /note="Description of Artificial Sequence: Synthetic peptide"
CAREGSSGWYGYVHHW

SEQ ID NO: 103 - protein, 6 aa, Artificial Sequence
  source: /note="Description of Artificial Sequence: Synthetic peptide"
EDIYNG

SEQ ID NO: 104 - protein, 3 aa, Artificial Sequence
  source: /note="Description of Artificial Sequence: Synthetic peptide"
NAN

SEQ ID NO: 105 - protein, 11 aa, Artificial Sequence
  source: /note="Description of Artificial Sequence: Synthetic peptide"
CQQYYDYPPTF

SEQ ID NO: 106 - DNA, 369 bp, Artificial Sequence
  source: /note="Description of Artificial Sequence: Synthetic polynucleotide"
caggtgcagctgcaggagtcgggcccaggactggtgaagccttcggagaccctgtccctcacctgcactgtctctggtggctccttcagcagtagtagttactactggggctggatccgccagccccctgggaaggggctggagtggattgggatcttctattatagtgggaccacctactacaacccgtccctcaagagtcgagtcaccatatccgcacacacgtccaagagccagttctccctgaagctgagctctgtgaccgccgcagacacggctgtgtattactgtgcgagagggggagaatattttgaccggttactcccctttgactactggggccagggaaccctggtcaccgtctcgagt

SEQ ID NO: 107 - DNA, 321 bp, Artificial Sequence
  source: /note="Description of Artificial Sequence: Synthetic polynucleotide"
gaaattgtgatgacgcagtctccatccttcctgtctgcatctgtaggagacagagtcaccatcacttgccgggccagtcagggcattagcagttatttagcctggtatcagcaaaaaccagggaaagcccctaagctcctgatctatgctgcatccactttggaaagtggggtcccatcaaggttcagcggcagtggatctgggacagaattcactctcacaatcagcagcctgcagcctgaagattttgcaacttattactgtcaacagcttaatagttacccattcactttcggccctgggaccaaagtggatatcaaa

SEQ ID NO: 108 - protein, 123 aa, Artificial Sequence
  source: /note="Description of Artificial Sequence: Synthetic polypeptide"
QVQLQESGPGLVKPSETLSLTCTVSGGSFSSSSYYWGWIRQPPGKGLEWIGIFYYSGTTYYNPSLKSRVTISAHTSKSQFSLKLSSVTAADTAVYYCARGGEYFDRLLPFDYWGQGTLVTVSS

SEQ ID NO: 109 - protein, 107 aa, Artificial Sequence
  source: /note="Description of Artificial Sequence: Synthetic polypeptide"
EIVMTQSPSFLSASVGDRVTITCRASQGISSYLAWYQQKPGKAPKLLIYAASTLESGVPSRFSGSGSGTEFTLTISSLQPEDFATYYCQQLNSYPFTFGPGTKVDIK

SEQ ID NO: 110 - protein, 10 aa, Artificial Sequence
  source: /note="Description of Artificial Sequence: Synthetic peptide"
GGSFSSSSYY

SEQ ID NO: 111 - protein, 7 aa, Artificial Sequence
  source: /note="Description of Artificial Sequence: Synthetic peptide"
FYYSGTT

SEQ ID NO: 112 - protein, 17 aa, Artificial Sequence
  source: /note="Description of Artificial Sequence: Synthetic peptide"
CARGGEYFDRLLPFDYW

SEQ ID NO: 113 - protein, 6 aa, Artificial Sequence
  source: /note="Description of Artificial Sequence: Synthetic peptide"
QGISSY

SEQ ID NO: 114 - protein, 3 aa, Artificial Sequence
  source: /note="Description of Artificial Sequence: Synthetic peptide"
AAS

SEQ ID NO: 115 - protein, 11 aa, Artificial Sequence [sequence omitted]

SEQ ID NO: 116 - DNA, 351 bp, Artificial Sequence
  source: /note="Description of Artificial Sequence: Synthetic polynucleotide"
caggtgcagctggtggagtctgggggaggcttggtacagccgggggggtccctgagactctcctgtacagcctctggattcacctttagcagctatgccatgagctgggtccgccaggctccagggaaggggctggagtgggtctcagctattggtggtagtggtggtagcacatactacgcagactccgtgaagggccggttcaccatctccagagacaattccaagaacacgctgtatctgcaaatgaacagcctgagagccgaggacacggccgtatattactgtgtgaaagatggggcaggaggctttgactactggggccagggaaccctggtcaccgtctcgagt

SEQ ID NO: 117 - DNA, 321 bp, Artificial Sequence
  source: /note="Description of Artificial Sequence: Synthetic polynucleotide"
gatattgtgatgacgcagtcttcatcctccctgtctgcatctgtaggagacagagtcaccatcacttgccgggcaagtcagggcattataaatcatttaggctggtatcagcataaaccagggaaagcccctaatcgcctaatctatgctgcatccagtttgcaaagtggggtcccatcaaggttcagcggcagtggatctgggacagaattcactctcacaatcagcagcctgcagcctgaagattttgcaacttattactgtctacggcataatagttaccctccgacgttcggccaagggaccaaggtggaaatcaag

SEQ ID NO: 118 - protein, 117 aa, Artificial Sequence
  source: /note="Description of Artificial Sequence: Synthetic polypeptide"
QVQLVESGGGLVQPGGSLRLSCTASGFTFSSYAMSWVRQAPGKGLEWVSAIGGSGGSTYYADSVKGRFTISRDNSKNTLYLQMNSLRAEDTAVYYCVKDGAGGFDYWGQGTLVTVSS

SEQ ID NO: 119 - protein, 107 aa, Artificial Sequence
  source: /note="Description of Artificial Sequence: Synthetic polypeptide"
DIVMTQSSSSLSASVGDRVTITCRASQGIINHLGWYQHKPGKAPNRLIYAASSLQSGVPSRFSGSGSGTEFTLTISSLQPEDFATYYCLRHNSYPPTFGQGTKVEIK

SEQ ID NO: 120 - protein, 8 aa, Artificial Sequence
  source: /note="Description of Artificial Sequence: Synthetic peptide"
GFTFSSYA

SEQ ID NO: 121 - protein, 8 aa, Artificial Sequence
  source: /note="Description of Artificial Sequence: Synthetic peptide"
IGGSGGST

SEQ ID NO: 122 - protein, 12 aa, Artificial Sequence
  source: /note="Description of Artificial Sequence: Synthetic peptide"
CVKDGAGGFDYW

SEQ ID NO: 123 - protein, 6 aa, Artificial Sequence
  source: /note="Description of Artificial Sequence: Synthetic peptide"
QGIINH

SEQ ID NO: 124 - protein, 3 aa, Artificial Sequence
  source: /note="Description of Artificial Sequence: Synthetic peptide"
AAS

SEQ ID NO: 125 - protein, 11 aa, Artificial Sequence
  source: /note="Description of Artificial Sequence: Synthetic peptide"
CLRHNSYPPTF

SEQ ID NO: 126 - DNA, 366 bp, Artificial Sequence
  source: /note="Description of Artificial Sequence: Synthetic polynucleotide"
caggtgcagctacagcagtcgggcccaggactggtgaagccttcacagaccctgtccctcacctgcactgtctctggtggctccatcaacagtggtggtcactactggagctggatccgccagcacccagggaggggcctggagtggattgggtacatctattacagtgggagcatctactacaacccgtccctcaagagtcgacttaccatatcagtagacacgtctaagaaccagttctccctgaagctgagctctgtgactgccgcggacacggccgtgtattactgtgcgagttattactatgccagtagtggtgatgcttttgatatctggggccaagggacaatggtcaccgtctcgagt

SEQ ID NO: 127 - DNA, 321 bp, Artificial Sequence
  source: /note="Description of Artificial Sequence: Synthetic polynucleotide"
gaaacgacactcacgcagtctccagccaccctgtctttgtctccaggggaaagagccaccctctcctgcagggccagtcagagtgttagcagctacttagcctggtaccaacagaaacctggccaggctcccaggctcctcatctatgatgcatccaacagggccactggcatcccagccaggttcagtggcagtgggtctgggacagacttcactctcaccatcagcagcctagagcctgaagattttgcagtttattactgtcagcagcgtagcaactggcctccgacgttcggccaagggaccaaggtggaaatcaaa

SEQ ID NO: 128 - protein, 122 aa, Artificial Sequence
  source: /note="Description of Artificial Sequence: Synthetic polypeptide"
QVQLQQSGPGLVKPSQTLSLTCTVSGGSINSGGHYWSWIRQHPGRGLEWIGYIYYSGSIYYNPSLKSRLTISVDTSKNQFSLKLSSVTAADTAVYYCASYYYASSGDAFDIWGQGTMVTVSS

SEQ ID NO: 129 - protein, 107 aa, Artificial Sequence
  source: /note="Description of Artificial Sequence: Synthetic polypeptide"
ETTLTQSPATLSLSPGERATLSCRASQSVSSYLAWYQQKPGQAPRLLIYDASNRATGIPARFSGSGSGTDFTLTISSLEPEDFAVYYCQQRSNWPPTFGQGTKVEIK

SEQ ID NO: 130 - protein, 10 aa, Artificial Sequence
  source: /note="Description of Artificial Sequence: Synthetic peptide"
GGSINSGGHY

SEQ ID NO: 131 - protein, 7 aa, Artificial Sequence
  source: /note="Description of Artificial Sequence: Synthetic peptide"
IYYSGSI

SEQ ID NO: 132 - protein, 16 aa, Artificial Sequence
  source: /note="Description of Artificial Sequence: Synthetic peptide"
CASYYYASSGDAFDIW

SEQ ID NO: 133 - protein, 6 aa, Artificial Sequence
  source: /note="Description of Artificial Sequence: Synthetic peptide"
QSVSSY

SEQ ID NO: 134 - protein, 3 aa, Artificial Sequence
  source: /note="Description of Artificial Sequence: Synthetic peptide"
DAS

SEQ ID NO: 135 - protein, 11 aa, Artificial Sequence [sequence omitted]

SEQ ID NO: 136 - DNA, 372 bp, Artificial Sequence
  source: /note="Description of Artificial Sequence: Synthetic polynucleotide"
caggtgcagctgcaggagtctgggggaggcttggtacagccgggggggtccctgagactctcctgtacagcctctggattcacctttagtaattatgccatgagctgggtccgccaggctccagggaaggggctggagtgggtctcagctattagtggtcgtggtggtagcacattcttcgcagactccgtgaagggccggttcaccatctccagagacaattccaagagcacgctgtatctgcaaacgaacagcctgagagccgaggacacggccgtatattactgtgcgaaagggggcccgttgtataactggaacgacggtgatggttttgatatctggggccaagggaccacggtcacagtctcgagt

SEQ ID NO: 137 - DNA, 324 bp, Artificial Sequence
  source: /note="Description of Artificial Sequence: Synthetic polynucleotide"
gaaattgtgttgacgcagtctccagccaccctgtctgtgtctccaggggaaagagccaccctctcctgcagggccagtcagagtgttagcagcaacttagcctggtaccagcagaaacctggccaggctcccaggctcctcatctatggtgcatccaccagggccactggtatcccagccaggttcagtggcactgggtctgggacagagttcactctcaccatcagcagcctgcagtctgaagattttgcactttattactgtcagcagtatgataactggcctccgtggacgttcggccaagggaccaaggtggaaatcaaa

SEQ ID NO: 138 - protein, 124 aa, Artificial Sequence
  source: /note="Description of Artificial Sequence: Synthetic polypeptide"
QVQLQESGGGLVQPGGSLRLSCTASGFTFSNYAMSWVRQAPGKGLEWVSAISGRGGSTFFADSVKGRFTISRDNSKSTLYLQTNSLRAEDTAVYYCAKGGPLYNWNDGDGFDIWGQGTTVTVSS

SEQ ID NO: 139 - protein, 108 aa, Artificial Sequence
  source: /note="Description of Artificial Sequence: Synthetic polypeptide"
EIVLTQSPATLSVSPGERATLSCRASQSVSSNLAWYQQKPGQAPRLLIYGASTRATGIPARFSGTGSGTEFTLTISSLQSEDFALYYCQQYDNWPPWTFGQGTKVEIK

SEQ ID NO: 140 - protein, 8 aa, Artificial Sequence
  source: /note="Description of Artificial Sequence: Synthetic peptide"
GFTFSNYA

SEQ ID NO: 141 - protein, 8 aa, Artificial Sequence
  source: /note="Description of Artificial Sequence: Synthetic peptide"
ISGRGGST

SEQ ID NO: 142 - protein, 19 aa, Artificial Sequence
  source: /note="Description of Artificial Sequence: Synthetic peptide"
CAKGGPLYNWNDGDGFDIW

SEQ ID NO: 143 - protein, 6 aa, Artificial Sequence
  source: /note="Description of Artificial Sequence: Synthetic peptide"
QSVSSN

SEQ ID NO: 144 - protein, 3 aa, Artificial Sequence
  source: /note="Description of Artificial Sequence: Synthetic peptide"
GAS

SEQ ID NO: 145 - protein, 12 aa, Artificial Sequence [sequence omitted]

SEQ ID NO: 146 - DNA, 357 bp, Artificial Sequence
  source: /note="Description of Artificial Sequence: Synthetic polynucleotide"
caggtgcagctgcaggagtctgggggaggcttggtcaagcctggagggtccctgagactctcctgtgcagcctctggattcaccttcagtgactactacatgacctggatccgccaggctccagggaaggggctggagtggatttcatacattagtggtggtggtggttccatatactacgcagactctgtgaagggccgattcaccatctccagggacaacgccaagaactcactgtatctgcaaatgaacagcctgagagccgaggacacggccgtttatttctgtgcgagagggaactggggatcggcggctcttgatatctggggccaagggacaatggtcacggtctcgagt

SEQ ID NO: 147 - DNA, 321 bp, Artificial Sequence
  source: /note="Description of Artificial Sequence: Synthetic polynucleotide"
gaaattgtgttgacgcagtctccatcctcactgtctgcatctgtaggagacagagtcaccatcacttgtcgggcgagtcagggcattaacaattatttagcctggtttcagcagaaaccagggagagcccctaagtccctgatctatgctgcatccagtttgcaaagtggggtcccatcgaagttcagcggcagtggatctgggacagatttcactctcaccatcagcagcctgcagcctgaagattttgcaacttattactgccaacagtataatagttaccctccaactctcggccctgggaccaacgtggatatcaaa

SEQ ID NO: 148 - protein, 119 aa, Artificial Sequence
  source: /note="Description of Artificial Sequence: Synthetic polypeptide"
QVQLQESGGGLVKPGGSLRLSCAASGFTFSDYYMTWIRQAPGKGLEWISYISGGGGSIYYADSVKGRFTISRDNAKNSLYLQMNSLRAEDTAVYFCARGNWGSAALDIWGQGTMVTVSS

SEQ ID NO: 149 - protein, 107 aa, Artificial Sequence
  source: /note="Description of Artificial Sequence: Synthetic polypeptide"
EIVLTQSPSSLSASVGDRVTITCRASQGINNYLAWFQQKPGRAPKSLIYAASSLQSGVPSKFSGSGSGTDFTLTISSLQPEDFATYYCQQYNSYPPTLGPGTNVDIK

SEQ ID NO: 150 - protein, 8 aa, Artificial Sequence
  source: /note="Description of Artificial Sequence: Synthetic peptide"
GFTFSDYY

SEQ ID NO: 151 - protein, 8 aa, Artificial Sequence
  source: /note="Description of Artificial Sequence: Synthetic peptide"
ISGGGGSI

SEQ ID NO: 152 - protein, 14 aa, Artificial Sequence
  source: /note="Description of Artificial Sequence: Synthetic peptide"
CARGNWGSAALDIW

SEQ ID NO: 153 - protein, 6 aa, Artificial Sequence
  source: /note="Description of Artificial Sequence: Synthetic peptide"
QGINNY

SEQ ID NO: 154 - protein, 3 aa, Artificial Sequence
  source: /note="Description of Artificial Sequence: Synthetic peptide"
AAS

SEQ ID NO: 155 - protein, 11 aa, Artificial Sequence
  source: /note="Description of Artificial Sequence: Synthetic peptide"
CQQYNSYPPTL

SEQ ID NO: 156 - DNA, 351 bp, Artificial Sequence
  source: /note="Description of Artificial Sequence: Synthetic polynucleotide"
caggtgcagctggtggagtctgggggaggcttggtacagccgggggggtccctgagactctcctgtacagcctctggattcacctttagcagctatgccatgagctgggtccgccaggctccagggaaggggctggagtgggtctcagctattggtggtagtggtggtagcgcatactacgcagactccgtgaagggccggttcaccatctccagagacaattccaagaacacgctgtatctgcaaatgaacagcctgagagccgaggacacggccgtatattactgtgtgaaagatggggcaggaggctttgactactggggccagggcaccctggtcaccgtctcgagt

SEQ ID NO: 157 - DNA, 321 bp, Artificial Sequence
  source: /note="Description of Artificial Sequence: Synthetic polynucleotide"
gacatccagttgacccagtccccatcctccctgtctgcatctgtaggagacagagtcaccatcacttgccgggcaagtcagggcattagaaatcatttaggctggtatcagcagaaaccagggaaagcccctaagcgcctaatctatgctgcatccagtttgcaaagtggggtcccatcaaggttcagcggcagtggatctgggacagaattcactctcacaatcagcagcctgcagcctgaagattttgcaacttattactgtctacagcataatagttaccctccgacgttcggccaagggaccaaggtggaaatcaag

SEQ ID NO: 158 - protein, 117 aa, Artificial Sequence
  source: /note="Description of Artificial Sequence: Synthetic polypeptide"
QVQLVESGGGLVQPGGSLRLSCTASGFTFSSYAMSWVRQAPGKGLEWVSAIGGSGGSAYYADSVKGRFTISRDNSKNTLYLQMNSLRAEDTAVYYCVKDGAGGFDYWGQGTLVTVSS

SEQ ID NO: 159 - protein, 107 aa, Artificial Sequence
  source: /note="Description of Artificial Sequence: Synthetic polypeptide"
DIQLTQSPSSLSASVGDRVTITCRASQGIRNHLGWYQQKPGKAPKRLIYAASSLQSGVPSRFSGSGSGTEFTLTISSLQPEDFATYYCLQHNSYPPTFGQGTKVEIK

SEQ ID NO: 160 - protein, 8 aa, Artificial Sequence
  source: /note="Description of Artificial Sequence: Synthetic peptide"
GFTFSSYA

SEQ ID NO: 161 - protein, 8 aa, Artificial Sequence
  source: /note="Description of Artificial Sequence: Synthetic peptide"
IGGSGGSA

SEQ ID NO: 162 - protein, 12 aa, Artificial Sequence
  source: /note="Description of Artificial Sequence: Synthetic peptide"
CVKDGAGGFDYW

SEQ ID NO: 163 - protein, 6 aa, Artificial Sequence
  source: /note="Description of Artificial Sequence: Synthetic peptide"
QGIRNH

SEQ ID NO: 164 - protein, 3 aa, Artificial Sequence
  source: /note="Description of Artificial Sequence: Synthetic peptide"
AAS

SEQ ID NO: 165 - protein, 11 aa, Artificial Sequence [sequence omitted]

SEQ ID NO: 166 - DNA, 354 bp, Artificial Sequence
  source: /note="Description of Artificial Sequence: Synthetic polynucleotide"
cagatgcagctacagcagtctgggggaggcttggtacagccgggggggtccctgagactctcctgtgcagcctctggattcaccgttagcagctatgccatgagctgggtccgccaggctctagggaaggggctggagtgggtctcaggtattagtggtagtggtggtagcacatactacgcagactccgtgaagggccggttcaccatctccagagacaattccaagaatacgctgtatctgcaaatgaacagcctgagagccgaggacacggccgtatattactgtgcgaagatagtgggagctacccactttgactactggggccagggaaccctggtcacggtctcgagt

SEQ ID NO: 167 - DNA, 339 bp, Artificial Sequence
  source: /note="Description of Artificial Sequence: Synthetic polynucleotide"
gaaattgtgatgacacagtctccagactccctggctgtgtctctgggcgagagggccaccatcaactgcaagtccagccagagtgttttatacagctccaacaataagaactacttagcttggtaccagcagaaaccaggacagcctcctaagctgctcatttactgggcatctacccgggaatccggggtccctgaccgattcagtggcagcgggtctgggacagatttcactctcaccatcagcagcctgcaggctgaagatgtggcagtttattactgtcagcaatattatagtggtccgatcaccttcggccaagggacacgactggagattaag

SEQ ID NO: 168 - protein, 118 aa, Artificial Sequence
  source: /note="Description of Artificial Sequence: Synthetic polypeptide"
QMQLQQSGGGLVQPGGSLRLSCAASGFTVSSYAMSWVRQALGKGLEWVSGISGSGGSTYYADSVKGRFTISRDNSKNTLYLQMNSLRAEDTAVYYCAKIVGATHFDYWGQGTLVTVSS

SEQ ID NO: 169 - protein, 113 aa, Artificial Sequence
  source: /note="Description of Artificial Sequence: Synthetic polypeptide"
EIVMTQSPDSLAVSLGERATINCKSSQSVLYSSNNKNYLAWYQQKPGQPPKLLIYWASTRESGVPDRFSGSGSGTDFTLTISSLQAEDVAVYYCQQYYSGPITFGQGTRLEIK

SEQ ID NO: 170 - protein, 8 aa, Artificial Sequence
  source: /note="Description of Artificial Sequence: Synthetic peptide"
GFTVSSYA

SEQ ID NO: 171 - protein, 8 aa, Artificial Sequence
  source: /note="Description of Artificial Sequence: Synthetic peptide"
ISGSGGST

SEQ ID NO: 172 - protein, 13 aa, Artificial Sequence
  source: /note="Description of Artificial Sequence: Synthetic peptide"
CAKIVGATHFDYW

SEQ ID NO: 173 - protein, 12 aa, Artificial Sequence
  source: /note="Description of Artificial Sequence: Synthetic peptide"
QSVLYSSNNKNY

SEQ ID NO: 174 - protein, 3 aa, Artificial Sequence
  source: /note="Description of Artificial Sequence: Synthetic peptide"
WAS

SEQ ID NO: 175 - protein, 11 aa, Artificial Sequence [sequence omitted]

SEQ ID NO: 176 - DNA, 366 bp, Artificial Sequence
  source: /note="Description of Artificial Sequence: Synthetic polynucleotide"
caggtgcagctggtggagtcgggcccaggactggtgaagccttcacagaccctgtccctcacctgcactgtctctggtggctccatcaacagtggtggttactactggagctggatccgccagcacccagggaagggcctggagtggattgggtacatctattacagtgggagcatctactacaacccgtccctcaggagtcgacttaccatatcagtagacacgtctaagaaccagttctccctgaagctgagctctgtgactgccgcggacacggccgtttattactgtgcgactccttattactatggttcggggagttatggggactactggggccagggcaccctggtcactgtctcgagt

SEQ ID NO: 177 - DNA, 321 bp, Artificial Sequence
  source: /note="Description of Artificial Sequence: Synthetic polynucleotide"
gacatccagatgacccagtctccagccaccctgtctttgtctccaggggaaagagccaccctctcctgcagggccagtcagagtgttaacaactacttagcctggtaccaacagaaacctggccaggctcccaggctcctcatctatgatgcatccaacagggccactggcatcccagccaggttcagtggcagtgggtctgggacagacttcactctcaccatcagcagcctagagcctgaagattttgcagtttattactgtcagcagcgtagcaactggcccatcaccttcggccaagggacacgactggagattaaa

SEQ ID NO: 178 - protein, 122 aa, Artificial Sequence
  source: /note="Description of Artificial Sequence: Synthetic polypeptide"
QVQLVESGPGLVKPSQTLSLTCTVSGGSINSGGYYWSWIRQHPGKGLEWIGYIYYSGSIYYNPSLRSRLTISVDTSKNQFSLKLSSVTAADTAVYYCATPYYYGSGSYGDYWGQGTLVTVSS

SEQ ID NO: 179 - protein, 107 aa, Artificial Sequence
  source: /note="Description of Artificial Sequence: Synthetic polypeptide"
DIQMTQSPATLSLSPGERATLSCRASQSVNNYLAWYQQKPGQAPRLLIYDASNRATGIPARFSGSGSGTDFTLTISSLEPEDFAVYYCQQRSNWPITFGQGTRLEIK

SEQ ID NO: 180 - protein, 10 aa, Artificial Sequence
  source: /note="Description of Artificial Sequence: Synthetic peptide"
GGSINSGGYY

SEQ ID NO: 181 - protein, 7 aa, Artificial Sequence
  source: /note="Description of Artificial Sequence: Synthetic peptide"
IYYSGSI

SEQ ID NO: 182 - protein, 16 aa, Artificial Sequence
  source: /note="Description of Artificial Sequence: Synthetic peptide"
CATPYYYGSGSYGDYW

SEQ ID NO: 183 - protein, 6 aa, Artificial Sequence
  source: /note="Description of Artificial Sequence: Synthetic peptide"
QSVNNY

SEQ ID NO: 184 - protein, 3 aa, Artificial Sequence
  source: /note="Description of Artificial Sequence: Synthetic peptide"
DAS

SEQ ID NO: 185 - protein, 11 aa, Artificial Sequence [sequence omitted]

SEQ ID NO: 186 - DNA, 363 bp, Artificial Sequence
  source: /note="Description of Artificial Sequence: Synthetic polynucleotide"
cagatgcagctgcaggagtcgggcccaggactggtgaagccttctcagaccctgtccctcacctgcactgtgtctggtggctccatcagcagtgttggttactactggaactggatccgccagcacccagggaagggcctggagttcattgggtacatctattacagtgggagcatctactacaatccgtccctcaagagtcgagttaccatatccgtagacacgtctaagaaccagttctccctgaagctgagctctgtgactgccgcggacacggccctatattactgtgcgagcgtcggtatagtgggagcctcctactttgagtactggggccagggaaccctggtcacagtctcgagt

SEQ ID NO: 187 - DNA, 321 bp, Artificial Sequence
  source: /note="Description of Artificial Sequence: Synthetic polynucleotide"
gaaattgtgatgacacagtctccagccaccctgtctttgtctccaggggaaagagccaccctctcctgcagggccagtcagagtgttagcagctacttagcctggtaccaacagaaacctggccaggctcccaggctcctcatctatgatgcatccaacagggccactggcatcccagccaggttcagtggcagtgggtctgggacagacttcactctcaccatcagcagcctagagcctgaagattttgcagtttattactgtcagcagcgtagcaactggcctatcaccttcggccaagggacacgactggagatcaag

SEQ ID NO: 188 - protein, 121 aa, Artificial Sequence
  source: /note="Description of Artificial Sequence: Synthetic polypeptide"
QMQLQESGPGLVKPSQTLSLTCTVSGGSISSVGYYWNWIRQHPGKGLEFIGYIYYSGSIYYNPSLKSRVTISVDTSKNQFSLKLSSVTAADTALYYCASVGIVGASYFEYWGQGTLVTVSS

SEQ ID NO: 189 - protein, 107 aa, Artificial Sequence
  source: /note="Description of Artificial Sequence: Synthetic polypeptide"
EIVMTQSPATLSLSPGERATLSCRASQSVSSYLAWYQQKPGQAPRLLIYDASNRATGIPARFSGSGSGTDFTLTISSLEPEDFAVYYCQQRSNWPITFGQGTRLEIK

SEQ ID NO: 190 - protein, 10 aa, Artificial Sequence
  source: /note="Description of Artificial Sequence: Synthetic peptide"
GGSISSVGYY

SEQ ID NO: 191 - protein, 7 aa, Artificial Sequence
  source: /note="Description of Artificial Sequence: Synthetic peptide"
IYYSGSI

SEQ ID NO: 192 - protein, 15 aa, Artificial Sequence
  source: /note="Description of Artificial Sequence: Synthetic peptide"
CASVGIVGASYFEYW

SEQ ID NO: 193 - protein, 6 aa, Artificial Sequence
  source: /note="Description of Artificial Sequence: Synthetic peptide"
QSVSSY

SEQ ID NO: 194 - protein, 3 aa, Artificial Sequence
  source: /note="Description of Artificial Sequence: Synthetic peptide"
DAS

SEQ ID NO: 195 - protein, 11 aa, Artificial Sequence [sequence omitted]

SEQ ID NO: 196 - DNA, 354 bp, Artificial Sequence
  source: /note="Description of Artificial Sequence: Synthetic polynucleotide"
caggtgcagctggtggagtctgggggaggcttggttcggcctggggggtccctgagactctcctgtgcagtctctggattcacctttagcagctatgccatgagctgggtccgccaggctccagggaaggggctggagtgggtctcaggtattagtggtagtggtggtagcacatacaacgcagactccgtgaagggccggttcaccatctccagagacaattccaagaacacgctgtatcttcaaatgaacagcctgagagccgaggacacggccgtatattactgtgcgaaaatttttgggtcctactactttgactactggggccagggaaccctggtcaccgtctcgagt

SEQ ID NO: 197 - DNA, 339 bp, Artificial Sequence
  source: /note="Description of Artificial Sequence: Synthetic polynucleotide"
gaaattgtgatgacacagtctccagactccctggctgtgtctctgggcgagagggccaccatcaactgcaagtccagccagagtgttttatacagctccaataataagaactacttagcttggtaccagcagaaatcaggacagcctcctaagctgctcatttactgggcatctacccgggaatccggggtccctgaccgattcagtggcagcgggtctgggacagatttcactctcaccatcagcagcctgcaggctgaagatgtggcagtttattactgtcagcaatattatagtggtccaccgacgttcggccaagggaccaaggtggaaatcaaa

SEQ ID NO: 198 - protein, 118 aa, Artificial Sequence
  source: /note="Description of Artificial Sequence: Synthetic polypeptide"
QVQLVESGGGLVRPGGSLRLSCAVSGFTFSSYAMSWVRQAPGKGLEWVSGISGSGGSTYNADSVKGRFTISRDNSKNTLYLQMNSLRAEDTAVYYCAKIFGSYYFDYWGQGTLVTVSS

SEQ ID NO: 199 - protein, 113 aa, Artificial Sequence
  source: /note="Description of Artificial Sequence: Synthetic polypeptide"
EIVMTQSPDSLAVSLGERATINCKSSQSVLYSSNNKNYLAWYQQKSGQPPKLLIYWASTRESGVPDRFSGSGSGTDFTLTISSLQAEDVAVYYCQQYYSGPPTFGQGTKVEIK

SEQ ID NO: 200 - protein, 8 aa, Artificial Sequence
  source: /note="Description of Artificial Sequence: Synthetic peptide"
GFTFSSYA

SEQ ID NO: 201 - protein, 8 aa, Artificial Sequence
  source: /note="Description of Artificial Sequence: Synthetic peptide"
ISGSGGST

SEQ ID NO: 202 - protein, 13 aa, Artificial Sequence
  source: /note="Description of Artificial Sequence: Synthetic peptide"
CAKIFGSYYFDYW

SEQ ID NO: 203 - protein, 12 aa, Artificial Sequence
  source: /note="Description of Artificial Sequence: Synthetic peptide"
QSVLYSSNNKNY

SEQ ID NO: 204 - protein, 3 aa, Artificial Sequence
  source: /note="Description of Artificial Sequence: Synthetic peptide"
WAS

SEQ ID NO: 205 - protein, 11 aa, Artificial Sequence [sequence omitted]

SEQ ID NO: 206 - DNA, 354 bp, Artificial Sequence
  source: /note="Description of Artificial Sequence: Synthetic polynucleotide"
caggtccagctacagcagtctgggggaggcttggttcatcctggggggtccctaagactctcctgtgcagcctctggattcaccgttgacacctatgccatgacctgggtccgccaggctccagggaaggggctggagtgggtctcaggtattagcggtagtggtggtagcacatactacgcagactccgtgaagggccggttcaccatctccagagacaactccaagaacacgctgtatctgcaaatgaacagcctgagagacgaggacacggccgtatattactgtgcgaagatagtgggagttacccactttgactactggggccagggcaccctggtcacggtctcgagt

SEQ ID NO: 207 - DNA, 339 bp, Artificial Sequence
  source: /note="Description of Artificial Sequence: Synthetic polynucleotide"
gaaattgtgatgacgcagtctccagactccctggctgtgtctctgggcgagagggccaccatcaactgcaagtccagccagagtgttttatacaggtccaacaataagaactatttagcttggtaccagcagaaaccaggacagcctcctaagctgctcatttactgggcatctacccgggaatccggggtccctgaccgattcagtggcagcgggtctgggacagatttcactctcaccatcagcagcctgcaggctgaagatgtggcagtttattactgtcagcaatattatagtggtccgatcaccttcggccaagggacacgactggagattaag

SEQ ID NO: 208 - protein, 118 aa, Artificial Sequence
  source: /note="Description of Artificial Sequence: Synthetic polypeptide"
QVQLQQSGGGLVHPGGSLRLSCAASGFTVDTYAMTWVRQAPGKGLEWVSGISGSGGSTYYADSVKGRFTISRDNSKNTLYLQMNSLRDEDTAVYYCAKIVGVTHFDYWGQGTLVTVSS

SEQ ID NO: 209 - protein, 113 aa, Artificial Sequence
  source: /note="Description of Artificial Sequence: Synthetic polypeptide"
EIVMTQSPDSLAVSLGERATINCKSSQSVLYRSNNKNYLAWYQQKPGQPPKLLIYWASTRESGVPDRFSGSGSGTDFTLTISSLQAEDVAVYYCQQYYSGPITFGQGTRLEIK

SEQ ID NO: 210 - protein, 8 aa, Artificial Sequence
  source: /note="Description of Artificial Sequence: Synthetic peptide"
GFTVDTYA

SEQ ID NO: 211 - protein, 8 aa, Artificial Sequence
  source: /note="Description of Artificial Sequence: Synthetic peptide"
ISGSGGST

SEQ ID NO: 212 - protein, 13 aa, Artificial Sequence
  source: /note="Description of Artificial Sequence: Synthetic peptide"
CAKIVGVTHFDYW

SEQ ID NO: 213 - protein, 12 aa, Artificial Sequence
  source: /note="Description of Artificial Sequence: Synthetic peptide"
QSVLYRSNNKNY

SEQ ID NO: 214 - protein, 3 aa, Artificial Sequence
  source: /note="Description of Artificial Sequence: Synthetic peptide"
WAS

SEQ ID NO: 215 - protein, 11 aa, Artificial Sequence [sequence omitted]

SEQ ID NO: 216 - DNA, 369 bp, Artificial Sequence
  source: /note="Description of Artificial Sequence: Synthetic polynucleotide"
caggtcaccttgaaggagtcgggcccaggactggtgaagccttcacagaccctgtccctcacctgcactgtctctggtggctccatcagcagtggtggtcattactggagctggatccgccagcacccagggaagggcctggagtggattgggtacatctcttacagtgggagcacctactacaacccgtccctcaagagtcgacttaccatatcagtagacacgtctaagaaccagttctccctgaagctgagctctgtgactgccgcggacacggccgtgtattactgtgcgaccgcgtattacgatattttgactggttacccttttgactactggggccagggaaccctggtcacggtctcgagt

SEQ ID NO: 217 - DNA, 321 bp, Artificial Sequence
  source: /note="Description of Artificial Sequence: Synthetic polynucleotide"
gaaattgtgatgacacagtctccagccaccctgtctttgtctccaggggaaagagccaccctctcctgcagggccagtcagagtgttagcagctacttagcctggtaccaacagaaacctggccaggctcccaggctcctcatctatgatgcatccgacagggccactggcatcccagccaggttcagtggcagtgggtctgggacagacttcactctcaccatcagcagcctagagcctgaagattttgcagtttattactgtcagcagcgtagcaactggccgatcaccttcggccaagggacacgactggagatcaag

SEQ ID NO: 218 - protein, 123 aa, Artificial Sequence
  source: /note="Description of Artificial Sequence: Synthetic polypeptide"
QVTLKESGPGLVKPSQTLSLTCTVSGGSISSGGHYWSWIRQHPGKGLEWIGYISYSGSTYYNPSLKSRLTISVDTSKNQFSLKLSSVTAADTAVYYCATAYYDILTGYPFDYWGQGTLVTVSS

SEQ ID NO: 219 - protein, 107 aa, Artificial Sequence
  source: /note="Description of Artificial Sequence: Synthetic polypeptide"
EIVMTQSPATLSLSPGERATLSCRASQSVSSYLAWYQQKPGQAPRLLIYDASDRATGIPARFSGSGSGTDFTLTISSLEPEDFAVYYCQQRSNWPITFGQGTRLEIK

SEQ ID NO: 220 - protein, 10 aa, Artificial Sequence
  source: /note="Description of Artificial Sequence: Synthetic peptide"
GGSISSGGHY

SEQ ID NO: 221 - protein, 7 aa, Artificial Sequence
  source: /note="Description of Artificial Sequence: Synthetic peptide"
ISYSGST

SEQ ID NO: 222 - protein, 17 aa, Artificial Sequence
  source: /note="Description of Artificial Sequence: Synthetic peptide"
CATAYYDILTGYPFDYW

SEQ ID NO: 223 - protein, 6 aa, Artificial Sequence
  source: /note="Description of Artificial Sequence: Synthetic peptide"
QSVSSY

SEQ ID NO: 224 - protein, 3 aa, Artificial Sequence
  source: /note="Description of Artificial Sequence: Synthetic peptide"
DAS

SEQ ID NO: 225 - protein, 11 aa, Artificial Sequence [sequence omitted]

SEQ ID NO: 226 - DNA, 369 bp, Artificial Sequence
  source: /note="Description of Artificial Sequence: Synthetic polynucleotide"
caggtgcagctacagcagtcgggcccaggactggtgaagccttcacagaccctgtccctcacctgcactgtctctggtggctccatcagcagtggtggttactactggagctggatccgccagcacccagggaagggcctggagtggattgggtacatctcttatagtgggagtatctactacaacccgtccctcaagagtcgagttaccatatcagtagacacgtctaagaaccagttctccctgaagctgagctctgtgactgccacggacacggccgtgtattactgtgcgaccgcgtattacgatcttttgactggttacccttttgactactggggccagggaaccctggtcacggtctcgagt

SEQ ID NO: 227 - DNA, 321 bp, Artificial Sequence
  source: /note="Description of Artificial Sequence: Synthetic polynucleotide"
gaaattgtgatgacgcagtctccagccaccctgtctttgtctccaggggaaagagccaccctctcctgcagggccagtcagagtgttagcagctacttagcctggtaccaacagaaacctggccaggctcccaggctcctcatctatgatgcatccaacagggccactggcatcccagccaggttcagtggcagtgggtctgggacagacttcactctcaccatcagcagcctagagcctgaagattttgcagtttattactgtcagcagcgtagcaactggccgatcaccttcggccaagggacacgactggagattaag

SEQ ID NO: 228 - protein, 123 aa, Artificial Sequence
  source: /note="Description of Artificial Sequence: Synthetic polypeptide"
QVQLQQSGPGLVKPSQTLSLTCTVSGGSISSGGYYWSWIRQHPGKGLEWIGYISYSGSIYYNPSLKSRVTISVDTSKNQFSLKLSSVTATDTAVYYCATAYYDLLTGYPFDYWGQGTLVTVSS

SEQ ID NO: 229 - protein, 107 aa, Artificial Sequence; identical to SEQ ID NO: 189
  source: /note="Description of Artificial Sequence: Synthetic polypeptide"

SEQ ID NO: 230 - protein, 10 aa, Artificial Sequence
  source: /note="Description of Artificial Sequence: Synthetic peptide"
GGSISSGGYY

SEQ ID NO: 231 - protein, 7 aa, Artificial Sequence
  source: /note="Description of Artificial Sequence: Synthetic peptide"
ISYSGSI

SEQ ID NO: 232 - protein, 17 aa, Artificial Sequence
  source: /note="Description of Artificial Sequence: Synthetic peptide"
CATAYYDLLTGYPFDYW

SEQ ID NO: 233 - protein, 6 aa, Artificial Sequence
  source: /note="Description of Artificial Sequence: Synthetic peptide"
QSVSSY

SEQ ID NO: 234 - protein, 3 aa, Artificial Sequence
  source: /note="Description of Artificial Sequence: Synthetic peptide"
DAS

SEQ ID NO: 235 - protein, 11 aa, Artificial Sequence [sequence omitted]

SEQ ID NO: 236 - protein, 301 aa, Homo sapiens
MFSHLPFDCVLLLLLLLLTRSSEVEYRAEVGQNAYLPCFYTPAAPGNLVPVCWGKGACPVFECGNVVLRTDERDVNYWTSRYWLNGDFRKGDVSLTIENVTLADSGIYCCRIQIPGIMNDEKFNLKLVIKPAKVTPAPTRQRDFTAAFPRMLTTRGHGPAETQTLGSLPDINLTQISTLANELRDSRLANDLRDSGATIRIGIYIGAGICAGLALALIFGALIFKWYSHSKEKIQNLSLISLANLPPSGLANAVAEGIRSEENIYTIEENVYEVEEPNEYYCYVSSRQQPSQPLGCRFAMP

SEQ ID NO: 237 - protein, 302 aa, Macaca fascicularis
MFSHLPFDCVLLLLLLLLTRSSEVEYIAEVGQNAYLPCSYTPAPPGNLVPVCWGKGACPVFDCSNVVLRTDNRDVNDRTSGRYWLKGDFHKGDVSLTIENVTLADSGVYCCRIQIPGIMNDEKHNVKLVVIKPAKVTPAPTLQRDLTSAFPRMLTTGEHGPAETQTPGSLPDVNLTVSNFFCELQIFTLTNELRDSGATIRTAIYIAAGISAGLALALIFGALIFKWYSHSKEKTQNLSLISLANIPPSGLANAVAEGIRSEENIYTIEEDVYEVEEPNEYYCYVSSGQQPSQPLGCRVAMP

SEQ ID NO: 238 - protein, 281 aa, Mus musculus
MFSGLTLNCVLLLLQLLLARSLENAYVFEVGKNAYLPCSYTLSTPGALVPMCWGKGFCPWSQCTNELLRTDERNVTYQKSSRYQLKGDLNKGDVSLIIKNVTLDDHGTYCCRIQFPGLMNDKKLELKLDIKAAKVTPAQTAHGDSTTASPRTLTTERNGSETQTLVTLHNNNGTKISTWADEIKDSGETIRTAIHIGVGVSAGLTLALIIGVLILKWYSCKKKKLSSLSLITLANLPPGGLANAGAVRIRSEENIYTIEENVYEVENSNEYYCYVNSQQPS

SEQ ID NO: 239 - protein, 282 aa, Rattus norvegicus
MFSWLPFSCALLLLQPLPARSLENAYTAEVGKNAYLPCSYTVPAPGTLVPICWGKGSCPLLQCASVVLRTDETNVTYRKSRRYQLKGNFYKGDMSLTIKNVTLADSGTYCCRIQFPGPMNDEKLELKLSITEPAKVIPAGTAHGDSTTASPRTLTTEGSGSETQTLVTLHDNNGTKISTWADEIKDSGETIRTAVHIGVGVSAGLALALILGVLILKWYSSKKKKLQDLSLITLANSPPGGLVNAGAGRIRSEENIYTIEENIYEMENSNEYYCYVSSQQPS

SEQ ID NO: 240 - protein, 15 aa, Artificial Sequence
  source: /note="Description of Artificial Sequence: Synthetic peptide"
GGGGSGGGGSGGGGS